European Patent Specification EP 3 574 101 B1, published April 19, 2023. Title: Repair template linkage to endonucleases for genome engineering. Applicant: KWS SAAT SE. The sequence listing filed with the application follows.

SEQUENCE LISTING (56 sequences)

SEQ ID NO: 1 - protein, 7 aa, Artificial Sequence
  NLS of the SV40 virus large T-antigen
PKKKRKV

SEQ ID NO: 2 - protein, 16 aa, Artificial Sequence
  Nucleoplasmin bipartite NLS
KRPAATKKAGQAKKKK

SEQ ID NO: 3 - protein, 9 aa, Artificial Sequence
  c-myc NLS
PAAKRVKLD

SEQ ID NO: 4 - protein, 11 aa, Artificial Sequence
  c-myc NLS
RQRRNELKRSP

SEQ ID NO: 5 - protein, 38 aa, Artificial Sequence
  hRNPA1 M9 NLS
NQSSNFGPMKGGNFGGRSSGPYGGGGQYFAKPRNQGGY

SEQ ID NO: 6 - protein, 42 aa, Artificial Sequence
  IBB domain from importin-alpha
RMRIZFKNKGKDTAELRRRRVEVSVELRKAKKDEQILKRRNV

SEQ ID NO: 7 - protein, 8 aa, Artificial Sequence
  Sequence derived from myoma T protein
VSRKRPRP

SEQ ID NO: 8 - protein, 8 aa, Artificial Sequence
  Sequence derived from myoma T protein
PPKKARED

SEQ ID NO: 9 - protein, 8 aa, Artificial Sequence
  Sequence derived from human p53
  misc_feature (2)..(2): Xaa can be any naturally occurring amino acid
PXPKKKPL

SEQ ID NO: 10 - protein, 12 aa, Artificial Sequence
  Sequence derived from mouse c-abl IV
SALIKKKKKMAP

SEQ ID NO: 11 - protein, 5 aa, Artificial Sequence
  Sequence derived from influenza virus NS1
DRLRR

SEQ ID NO: 12 - protein, 7 aa, Artificial Sequence
  Sequence derived from influenza virus NS1
PKQKKRK

SEQ ID NO: 13 - protein, 10 aa, Artificial Sequence
  Sequence derived from Hepatitis virus delta antigen
RKLKKKIKKL

SEQ ID NO: 14 - protein, 10 aa, Artificial Sequence
  Sequence derived from mouse Mx1 protein
REKKKFLKRR

SEQ ID NO: 15 - protein, 20 aa, Artificial Sequence
  Sequence derived from human poly(ADP-ribose) polymerase
KRKGDEVDGVDEVAKKKSKK

SEQ ID NO: 16 - protein, 17 aa, Artificial Sequence
  Derived from steroid hormone receptors (human) glucocorticoid
RKCLQAGMNLEARKTKK

SEQ ID NO: 17 - protein, 11 aa, Artificial Sequence
  Sequence derived from HIV Tat
YGRKKRRQRRR

SEQ ID NO: 18 - protein, 5 aa, Artificial Sequence
  Sequence derived from HIV Tat
GRKKR

SEQ ID NO: 19 - protein, 923 aa, Artificial Sequence
  2NLS-NgAgo: WT NgAgo amended with N- and C-terminal sequences
MASSPKKKRKVMTVIDLDSTTTADELTSGHTYDISVTLTGVYDNTDEQHPRMSLAFEQDNGERRYITLWKNTTPKDVFTYDYATGSTYIFTNIDYEVKDGYENLTATYQTTVENATAQEVGTTDEDETFAGGEPLDHHLDDALNETPDDAETESDSGHVMTSFASRDQLPEWTLHTYTLTATDGAKTDTEYARRTLAYTVRQELYTDHDAAPVATDGLMLLTPEPLGETPLDLDCGVRVEADETRTLDYTTAKDRLLARELVEEGLKRSLWDDYLVRGIDEVLSKEPVLTCDEFDLHERYDLSVEVGHSGRAYLHINFRHRFVPKLTLADIDDDNIYPGLRVKTTYRPRRGHIVWGLRDECATDSLNTLGNQSVVAYHRNNQTPINTDLLDAIEAADRRVVETRRQGHGDDAVSFPQELLAVEPNTHQIKQFASDGFHQQARSKTRLSASRCSEKAQAFAERLDPVRLNGSTVEFSSEFFTGNNEQQLRLLYENGESVLTFRDGARGAHPDETFSKGIVNPPESFEVAVVLPEQQADTCKAQWDTMADLLNQAGAPPTRSETVQYDAFSSPESISLNVAGAIDPSEVDAAFVVLPPDQEGFADLASPTETYDELKKALANMGIYSQMAYFDRFRDAKIFYTRNVALGLLAAAGGVAFTTEHAMPGDADMFIGIDVSRSYPEDGASGQINIAATATAVYKDGTILGHSSTRPQLGEKLQSTDVRDIMKNAILGYQQVTGESPTHIVIHRDGFMNEDLDPATEFLNEQGVEYDIVEIRKQPQTRLLAVSDVQYDTPVKSIAAINQNEPRATVATFGAPEYLATRDGGGLPRPIQIERVAGETDIETLTRQVYLLSQSHIQVHNSTARLPITTAYADQASTHATKGYLVQTGAFESNVGFLKRPAATKKAGQAKKKKYPYDVPDYA

SEQ ID NO: 20 - protein, 1159 aa, Artificial sequence
  2NLS-NgAgo-mNeonGreen
MASSPKKKRKVMTVIDLDSTTTADELTSGHTYDISVTLTGVYDNTDEQHPRMSLAFEQDNGERRYITLWKNTTPKDVFTYDYATGSTYIFTNIDYEVKDGYENLTATYQTTVENATAQEVGTTDEDETFAGGEPLDHHLDDALNETPDDAETESDSGHVMTSFASRDQLPEWTLHTYTLTATDGAKTDTEYARRTLAYTVRQELYTDHDAAPVATDGLMLLTPEPLGETPLDLDCGVRVEADETRTLDYTTAKDRLLARELVEEGLKRSLWDDYLVRGIDEVLSKEPVLTCDEFDLHERYDLSVEVGHSGRAYLHINFRHRFVPKLTLADIDDDNIYPGLRVKTTYRPRRGHIVWGLRDECATDSLNTLGNQSVVAYHRNNQTPINTDLLDAIEAADRRVVETRRQGHGDDAVSFPQELLAVEPNTHQIKQFASDGFHQQARSKTRLSASRCSEKAQAFAERLDPVRLNGSTVEFSSEFFTGNNEQQLRLLYENGESVLTFRDGARGAHPDETFSKGIVNPPESFEVAVVLPEQQADTCKAQWDTMADLLNQAGAPPTRSETVQYDAFSSPESISLNVAGAIDPSEVDAAFVVLPPDQEGFADLASPTETYDELKKALANMGIYSQMAYFDRFRDAKIFYTRNVALGLLAAAGGVAFTTEHAMPGDADMFIGIDVSRSYPEDGASGQINIAATATAVYKDGTILGHSSTRPQLGEKLQSTDVRDIMKNAILGYQQVTGESPTHIVIHRDGFMNEDLDPATEFLNEQGVEYDIVEIRKQPQTRLLAVSDVQYDTPVKSIAAINQNEPRATVATFGAPEYLATRDGGGLPRPIQIERVAGETDIETLTRQVYLLSQSHIQVHNSTARLPITTAYADQASTHATKGYLVQTGAFESNVGFLKRPAATKKAGQAKKKKYPYDVPDYAMVSKGEEDNMASLPATHELHIFGSINGVDFDMVGQGTGNPNDGYEELNLKSTKGDLQFSPWILVPHIGYGFHQYLPYPDGMSPFQAAMVDGSGYQVHRTMQFEDGASLTVNYRYTYEGSHIKGEAQVKGTGFPADGPVMTNSLTAADWCRSKKTYPNDKTIISTFKWSYTTGNGKRYRSTARTTYTFAKPMAANYLKNQPMYVFRKTELKHSKTELNFKEWQKAFTDVMGMDELYK

SEQ ID NO: 21 - protein, 887 aa, Natronobacterium gregoryi
MTVIDLDSTTTADELTSGHTYDISVTLTGVYDNTDEQHPRMSLAFEQDNGERRYITLWKNTTPKDVFTYDYATGSTYIFTNIDYEVKDGYENLTATYQTTVENATAQEVGTTDEDETFAGGEPLDHHLDDALNETPDDAETESDSGHVMTSFASRDQLPEWTLHTYTLTATDGAKTDTEYARRTLAYTVRQELYTDHDAAPVATDGLMLLTPEPLGETPLDLDCGVRVEADETRTLDYTTAKDRLLARELVEEGLKRSLWDDYLVRGIDEVLSKEPVLTCDEFDLHERYDLSVEVGHSGRAYLHINFRHRFVPKLTLADIDDDNIYPGLRVKTTYRPRRGHIVWGLRDECATDSLNTLGNQSVVAYHRNNQTPINTDLLDAIEAADRRVVETRRQGHGDDAVSFPQELLAVEPNTHQIKQFASDGFHQQARSKTRLSASRCSEKAQAFAERLDPVRLNGSTVEFSSEFFTGNNEQQLRLLYENGESVLTFRDGARGAHPDETFSKGIVNPPESFEVAVVLPEQQADTCKAQWDTMADLLNQAGAPPTRSETVQYDAFSSPESISLNVAGAIDPSEVDAAFVVLPPDQEGFADLASPTETYDELKKALANMGIYSQMAYFDRFRDAKIFYTRNVALGLLAAAGGVAFTTEHAMPGDADMFIGIDVSRSYPEDGASGQINIAATATAVYKDGTILGHSSTRPQLGEKLQSTDVRDIMKNAILGYQQVTGESPTHIVIHRDGFMNEDLDPATEFLNEQGVEYDIVEIRKQPQTRLLAVSDVQYDTPVKSIAAINQNEPRATVATFGAPEYLATRDGGGLPRPIQIERVAGETDIETLTRQVYLLSQSHIQVHNSTARLPITTAYADQASTHATKGYLVQTGAFESNVGFL

SEQ ID NO: 22 - protein, 747 aa, Microcystis aeruginosa
MNYTAANTANSPIFLSEISSLTLKNSCLNCFQLNHQVTRKIGNRFSWQFSRKFPDVVVIFEDNCFWVLAKDEKSIPSLQQWKEALSDIQEVLREDIGDHYYSIHWLKDFQITALVTAQLAVRILKIFGKFSDPIVFPKDSQISENQVQVRREVNFWAEIINDTDPAICLTVDSSIVYSGDLEQFYENHPYRQDAVKLLVGLKVKDRETNGTAKIIRIAGRIGERREDLLTKATGSISRRKLEEAHLGQPVVAVQFGKNPQEYIYPLAALKPWVTDEDESLFQVNYGNLLKATKIFYAERQELLKLYKQEAQKALNNFGFQLREKSINSQEYPELFWTPSISIEQTPILFGQGERGEKREIIKGLSKGGVYKRHREYVDPARKIRLAILKPANLKVGDFREQLEKRLKLYKFETILPPENQINFSVEGLGFEKRARLEEAVDRLIGVEIPVDIALVFLPQEDRNADNTEEGSLYSWIKRKFLGRGVITQMIYEKTLNDKSNYKNILNQVVPGILAKLGNLPYVLAEPLEIADYFIGLDVGRMPKKNLPGSLNVCASVRLYGKQGEFVRCRVEDSLTEGEEIPQRILENCLPQAELKNQTVLIYRDGKFQGKEVENLLARARAINAKFILVECYKTGIPRLYNLQQKQINAPSKGLALALSNREVILITSQVSEQIGVPRPLRLKVHELGEQRNLKQLVDTTLKLTLLHYGSLKDPRLPIPLYGADIIAYRRLQGIYPSLLEDDCQFWL

SEQ ID NO: 23 - protein, 863 aa, Halogeometricum pallidum
MVKRYISFHLFPRIKLCGVYLCLRMNTKDDIAHKQPITIEVQVLKELDKPSPKMATRLLVADRAGNRFPLAIWKNNALSDYDWTIGQWYRLENARGNVFNGKQSLNGSSNMRATPLEASEEDETRADDVGRVDTILGNLSPNQAYLSLFPISRSFDTLSVYEYSIEAAEAFEDDPDTVTYQCAGRLRRITGAGVAYAGPMQIVSTRKLPDKLADPFSLSEPTERELKAADARDRHRIERLLKSLVKAAIDDSTYDPYQINRIRARTPAITAGDGLFEACYEFAARVDVMPSGDAFVGIEVRYHARSQVTADVYEDKTGELVGTIVEHDPERYNVSGTGRVVGFTDHYFTDALDELGGLSLADWYAQKDRVPEGVLEALREKNPRLVDIQYQEDEPAQIHVPELLRVAPRKEVVKELDPTFHRRWDREAKMLPDKRFRHAIEFVDHLGSLPDIDATVAPEPLGPSLSYMSTAVDREENLRFKDGRTATTPSSGIRSGVYQQPTSFDIAYVYPTESEQESKQFISNFENKLSRCHCEPTATRHVPYELGGELSYLAVINELESVDAVLAVVPPRNDDRIAAGDITDPYPEFKKGLGKQKVPSQMVVTENLDTRWVMNNTAMGLIAGAGGVPWRVDEMPGEADCFIGLDVTRDPETGQHLGASANVVYADGTVFASKTQTLQSGETFDEQSIIDVIKDVFQEFVRREGRSPEHIVIHRDGRLFEDADEIQAPFADSGVSIDILDIRKSGAPRIARYEDNSFKIDEKGRLFISQDDTHGFIATTGKPEFDDSDNLGTPKTLRVVRRAGDTPMLTLLKQVYWLSEAHIGSVSRSVRLPITTYYADRCAEHAREGYLLHGELIEGVPYL

SEQ ID NO: 24 - protein, 839 aa, Natrialba asiatica
MKTQDDIAHKQPITIEVQILKELDKPSPKMATRFLVADRDGNRFSLAIWKNNALSDYDWTIGQWYRLENARGNVFNGKQSLNGSSKMRATPLEASEEDETSTDDVGRVDTILGNMSPDQAYLSLFPISRSFDTLSVYEYSIEAAEAFEDAPDTVTYRCAGRLRRITGAGVAYAGSMRIVSTRKLPDKLADPFSLSEPTERELNATDARDRHRIERLLKSLVKAAIDDSTYDPYQINRIRARTPSITAGDGLFEACYEFAARVDVMPSGDAFVGIEVRYHTRSQVTADVYEDKTAELVGTIVEHDPERYNISGTGRVVGFTDHHFTDALDELGGLSLADWYAQKDRVPEGVLEALREKNPRLVDIQYQEDEPARIHVPDLLRVAPRKEVVKELDPAFHRRWDREAKMLPDKRFRHAIEFVDHLGSLPDIDATVAPEPLGPSLSYMSTAVDREKNLRFKDGRTATTPSSGIRSGVYQQPTSFDIAYVYPTESEQESKQFISNFENKLSQCQCEPTAARHVPYELGGELSYLAVINELESVDAVLAVVPPRDDDRITAGDITDPYPEFKKGLGKQKIPSQMIVTENLGTRWVMNNTAMGLIAGAGGVPWRVDEMPGEADCFIGLDVTRDPETGQHLGASANVVYADGTVFASKTQTLQSGETFDEQSIIDVIKDVFQEFVRREGRSPEHIVIHRDGRLFEDADEIQAPFADSGVSIDILDIRKSGAPRIAQYEDNSFKIDEKGRLFISQDDTHGFIATTGKPEFDDSDNLGTPKTLRVVRRAGDTPMLTLLKQVYWLSEAHVGSVSRSVRLPITTYYADRCAEHAREGYLLHGELIEGVPYL

SEQ ID NO: 25 - protein, 889 aa, Natronorubrum tibetense
MAVKTDIEDGKQIDISLRVTGTDEWDHDAIARKVQLEDVEGTPVELTVFHNNEIADFEWDDERWYVLENVVGNEYRGEMQLNPGYDLIVTPLDEPPAAAENGGAENTSATQSSESGDSGSSTEADQSAESESARESEVTSEPRPTADGGGELLHQQPLSEGNYLLQFELGDLPELTVHEYELRATGSGGINPDDFTNGIEGFTAKAANYYQSRINSPVTTADASRRRIYATEKLHGKISIHGYTVKPVHQGETTLEARSYTDDGPLQEFVKQDVKRAVAGRFEVSGIDSIIEPTPQRTANSGLFEAYRKYKCRIRVDADGTVICGVNVAYHLESTFSAADWVQRGHDIAEVTVEHDTDLYDSARTATVKEVIDMDYDDVLDGPGVPMSEYHEQHVEQDVINSMQAGDPIIADLQYGSDEDSIFPQLLEYCKVIPTFDQLGSVDDTFLDVIHNESRMEPEERFSVVTSFVDLLGPTPYFSFDPVPQPTNAGYREHKTPNTPNLRFGDGKTGFYGAGGLERKGYGIYKAPESFDIIALYPEDEEDDARPYVLSLLNKLADYDAGPTVFDQETYELGSEFHYSQHAQKASDYDAALIVVPDADKAAAADYDDPYPEFKRRLGQLGVPSQMISVDNLGNDNYRGNICSSLIGKAGGVPWRIDDVPGDVDAFVGLDVTYDHATKQHLGAAANVIMADGTILASEAVTKQAGETFDEDDVANVIKHVLEIFAEEEGRPPRHVVIHRDGKFYLDVENLVKRLDKARDLIQRFDLVEIRKSGNPRIAAYDESESRFDIADKGIAFHVHNGDHSYLTTTGGREGSPGTPRPLQIVKRHGSTDLDTLAEQTYWLSEAHVGSLSRSTRLPITTYYADKCADFAMKGYLTKGSVIRGVPYI

SEQ ID NO: 26 - protein, 847 aa, Natrinema pellirubrum
MPTQSDIEDGERIDIQVKVLSELDRPSEKMAKRLRVRDTDGNEFPLTIWKNNALCDFAWERGRWYELENARGNEFRGEKSLNGSSRLHADPVDNPIDSDRSQQSTTAESTDKQFDSLEDGLPYLSLFPIDREFETVDVYEYRIEADGPFDDDPMDATYTLAAYLRSCSDAAVTHAGIFSVIATNRLTNALPDPFELTDESRVTLRADDETDNECLVRLLQQVFKTAVDDETYETGRVDRIRTQDPVITGQDGLFEACLAYTARLEILPSGKAFVGIDISYHARSQVTVDKYVDRINASVDELIDTPVEHDPERYEKSGSGRLKGFADVTFTDPVDDFGNQSLADWYEQKGRISDDMLERLRSEDPQLVEIQYNPNSDETNLHVPQLLRVAPRKEIVKKLAPTFHRKWDRAAKMLPDDRFRKATRFVARLDSLSEVDAQIEPNPVGPNISFMSTEVDRSDNLRFGDDQTTTLPNNGLKRYGIYRRPSSLHLHYLVPERYTDEFASFREQLERQLATIGCSPDDISYDEYGLGNAINYNTTAAAVDDVDIVLAVVPAPDNDFIRNGTIDDPYPEFKKSLGKQTIPSQMVREDNLDDRWILRNTALGVIAGAGGVPWRVDEMPGDVDCFVGLDATRDPETGQFLGASANVVLSDGTVFVSKTQSLQSGETFDENAIVDVLKDVHREFVREEGKSPNNIVIHRDGRLFEDVDTILEPFDETDIDIDILDVRKSGAPRAAVYQDDQFQVDHKGRLFVAQSGDYGFLTTTGRPEFDEDDGLGTPRSLRIVRRAGETPMRTLLEQVYWLSESHVGSAQRSTRLPITTYYADRCAEHAREGYLVNGELIRGVPYL

SEQ ID NO: 27 - protein, 747 aa, Microcystis aeruginosa
MNYTETKTANSPIFLSEISSLTLNNNCLNCFKLNHQVTRKIGNRFSWQFSRKFPAVVVIFEDNCFWVLAKDEKLLPSPQQWKEALSDIQEVLREDIGDHYYSIHWLKDFQITALVTAQLAVRILKIFGKFSYPIVFPKDSQISENQVQVRREVNFWAEIINDTDPAICLTLESSIVYSGDLEQFYENHPYRQDAAKLLVGLKVKTIETNGTAKIIRIAGTIGERREELLTKATGSISRRKLEEAHLGQPVVAVQFGKNSQEYIYPLAALKPCMTDKDESLFQVNYGELLKETKIFYAERQERLKLYKQEAQNTLNNFGFRLGEKSINSREYPELFWNPSISLEQTPILFGKGERGEKIKTLKGLSKGGVYKRHREYLDPARKIRLAILKPANLKVGDFREQLEKRLELYKFETILPAENQINFSVEGVGFEKRARLEEAVDQLIRGEIPVDIALVFLPQEDRNADNTEEGSLYSWIKKKFLERRVMTQMIYEKTLNDKSNYKNILNQVVPGILAKLGNLPYVLAESLEIADYFIGLDVGRMPKKNLPGSLNVCASVRLYGKQGEFVRCRVEDSLTEGEEIPQRILENCLPQAELKNQTVLIYRDGKFQGKEVDNLLARARAINAKFILVECYKTGIPRLYNFEQKQINAPSKGLAFALSKREVILITSQVSEQIGVPRPLRLKVHELGDQVNLKQLVDTTLKLTLLHYGSLKEPRLPIPLYGADAIAYRRLQGICPSLLEDDCQFWL

SEQ ID NO: 28 - protein, 747 aa, Microcystis aeruginosa; identical to SEQ ID NO: 22

SEQ ID NO: 29 - protein, 735 aa, Synechococcus elongatus
MDLLSNLRRSSIVLNRFYVKSLSQSDLTAYEYRCIFKKTPELGDEKRLLASICYKLGAIAVRIGSNIITKEAVRPEKLQGHDWQLVQMGTKQLDCRNDAHRCALETFERKFLERDLSASSQTEVRKAAEGGLIWWVVGAKGIEKSGNGWEVHRGRRIDVSLDAEGNLYLEIDIHHRFYTPWTVHQWLEQYPEIPLSYVRNNYLDERHGFINWQYGRFTQERPQDILLDCLGMSLAEYHLNKGATEEEVQQSYVVYVKPISWRKGKLTAHLSRRLSPSLTMEMLAKVAEDSTVCDREKREIRAVFKSIKQSINQRLQEAQKTASWILTKTYGISSPAIALSCDGYLLPAAKLLAANKQPVSKTADIRNKGCAKIGETSFGYLNLYNNQLQYPLEVHKCLLEIANKNNLQLSLDQRRVLSDYPQDDLDQQMFWQTWSSQGIKTVLVVMPWDSHHDKQKIRIQAIQAGIATQFMVPLPKADKYKALNVTLGLLCKAGWQPIQLESVDHPEVADLIIGFDTGTNRELYYGTSAFAVLADGQSLGWELPAVQRGETFSGQAIWQTVSKLIIKFYQICQRYPQKLLLMRDGLVQEGEFQQTIELLKERKIAVDVISVRKSGAGRMGQEIYENGQLVYRDAAIGSVILQPAERSFIMVTSQPVSKTIGSIRPLRIVHEYGSTDLELLALQTYHLTQLHPASGFRSCRLPWVLHLADRSSKEFQRIGQISVLQNISRDKLIAV

SEQ ID NO: 30 - protein, 25 aa, Saccharomyces cerevisiae
MLSLRQSIRFFKPATRTLCSSRYLL

SEQ ID NO: 31 - protein, 33 aa, Homo sapiens
MLSALARPASAALRRSFSTSAQNNAKVAVLGAS

SEQ ID NO: 32 - protein, 23 aa, Arabidopsis thaliana
MHSRSALLYRFLRPASRCFSSSS

SEQ ID NO: 33 - protein, 424 aa, Agrobacterium tumefaciens
MPDRAQVIIRIVPGGGTKTLQQIINQLEYLSRKGKLELQRSARHLDIPVPPDQIRELAQSWVTEAGIYDESQSDDDRQQDLTTHIIVSFPAGTDQTAAYEASREWAAEMFGSGYGGGRYNYLTAYHVDRDHPHLHVVVNRRELLGHGWLKISRRHPQLNYDGLRKKMAEISLRHGIVLDATSRAERGIAERPITYAEHRRLERMQAQKIQFEDTDFDETSPEEDRRDLSQSFDPFRSDPSTGEPDRATRHDKQPLEQHARFQESAGSSIKADARIRVSLESERSAQPSASKIPVIGHFGIETSYVAEASVRKRSGIFGTSRPVTDVAMHTVKRQQRSKRRNDEEAGPSGANRKGLKAAQVDSEANVGEQDTRDDSNKAADPVSASIGTEQPEASPKRPRDRHDGELGGRKRARGNRRDDGRGGT

SEQ ID NO: 34 - DNA, 387 bp, Artificial sequence
  pET-MBP-mSA2
gcggaagcgggtatcaccggcacgtggtacaaccagcatggttctaccttcaccgttaccgcgggtgcggacggtaacctgaccggtcagtacgaaaaccgtgcgcagggcactggttgccagaactctccgtacaccctgaccggtcgttacaacggtaccaaactggaatggcgtgttgaatggaacaactctaccgaaaactgccactctcgtaccgaatggcgtggtcagtaccagggtggtgcggaagcgcgtatcaacacccagtggaacctgacctacgaaggtggttctggtccggcgaccgaacagggtcaggacaccttcaccaaagttaaaccgtctgcggcgtctggatccgactacaaggacgatgacgacaag

SEQ ID NO: 35 - protein, 1300 aa, Francisella tularensis subsp. novicida U112
MSIYQEFVNKYSLSKTLRFELIPQGKTLENIKARGLILDDEKRAKDYKKAKQIIDKYHQFFIEEILSSVCISEDLLQNYSDVYFKLKKSDDDNLQKDFKSAKDTIKKQISEYIKDSEKFKNLFNQNLIDAKKGQESDLILWLKQSKDNGIELFKANSDITDIDEALEIIKSFKGWTTYFKGFHENRKNVYSSNDIPTSIIYRIVDDNLPKFLENKAKYESLKDKAPEAINYEQIKKDLAEELTFDIDYKTSEVNQRVFSLDEVFEIANFNNYLNQSGITKFNTIIGGKFVNGENTKRKGINEYINLYSQQINDKTLKKYKMSVLFKQILSDTESKSFVIDKLEDDSDVVTTMQSFYEQIAAFKTVEEKSIKETLSLLFDDLKAQKLDLSKIYFKNDKSLTDLSQQVFDDYSVIGTAVLEYITQQIAPKNLDNPSKKEQELIAKKTEKAKYLSLETIKLALEEFNKHRDIDKQCRFEEILANFAAIPMIFDEIAQNKDNLAQISIKYQNQGKKDLLQASAEDDVKAIKDLLDQTNNLLHKLKIFHISQSEDKANILDKDEHFYLVFEECYFELANIVPLYNKIRNYITQKPYSDEKFKLNFENSTLANGWDKNKEPDNTAILFIKDDKYYLGVMNKKNNKIFDDKAIKENKGEGYKKIVYKLLPGANKMLPKVFFSAKSIKFYNPSEDILRIRNHSTHTKNGSPQKGYEKFEFNIEDCRKFIDFYKQSISKHPEWKDFGFRFSDTQRYNSIDEFYREVENQGYKLTFENISESYIDSVVNQGKLYLFQIYNKDFSAYSKGRPNLHTLYWKALFDERNLQDVVYKLNGEAELFYRKQSIPKKITHPAKEAIANKNKDNPKKESVFEYDLIKDKRFTEDKFFFHCPITINFKSSGANKFNDEINLLLKEKANDVHILSIDRGERHLAYYTLVDGKGNIIKQDTFNIIGNDRMKTNYHDKLAAIEKDRDSARKDWKKINNIKEMKEGYLSQVVHEIAKLVIEYNAIVVFEDLNFGFKRGRFKVEKQVYQKLEKMLIEKLNYLVFKDNEFDKTGGVLRAYQLTAPFETFKKMGKQTGIIYYVPAGFTSKICPVTGFVNQLYPKYESVSKSQEFFSKFDKICYNLDKGYFEFSFDYKNFGDKAAKGKWTIASFGSRLINFRNSDKNHNWDTREVYPTKELEKLLKDYSIEYGHGECIKAAICGESDKKFFAKLTSVLNTILQMRNSKTGTELDYLISPVADVNGNFFDSRQAPKNMPQDADANGAYHIGLKGLMLLGRIKNNQEGKKLNLVIKNEEYFEFVQNRNN

SEQ ID NO: 36 - protein, 1307 aa, Acidaminococcus sp. BV3L6
MTQFEGFTNLYQVSKTLRFELIPQGKTLKHIQEQGFIEEDKARNDHYKELKPIIDRIYKTYADQCLQLVQLDWENLSAAIDSYRKEKTEETRNALIEEQATYRNAIHDYFIGRTDNLTDAINKRHAEIYKGLFKAELFNGKVLKQLGTVTTTEHENALLRSFDKFTTYFSGFYENRKNVFSAEDISTAIPHRIVQDNFPKFKENCHIFTRLITAVPSLREHFENVKKAIGIFVSTSIEEVFSFPFYNQLLTQTQIDLYNQLLGGISREAGTEKIKGLNEVLNLAIQKNDETAHIIASLPHRFIPLFKQILSDRNTLSFILEEFKSDEEVIQSFCKYKTLLRNENVLETAEALFNELNSIDLTHIFISHKKLETISSALCDHWDTLRNALYERRISELTGKITKSAKEKVQRSLKHEDINLQEIISAAGKELSEAFKQKTSEILSHAHAALDQPLPTTLKKQEEKEILKSQLDSLLGLYHLLDWFAVDESNEVDPEFSARLTGIKLEMEPSLSFYNKARNYATKKPYSVEKFKLNFQMPTLASGWDVNKEKNNGAILFVKNGLYYLGIMPKQKGRYKALSFEPTEKTSEGFDKMYYDYFPDAAKMIPKCSTQLKAVTAHFQTHTTPILLSNNFIEPLEITKEIYDLNNPEKEPKKFQTAYAKKTGDQKGYREALCKWIDFTRDFLSKYTKTTSIDLSSLRPSSQYKDLGEYYAELNPLLYHISFQRIAEKEIMDAVETGKLYLFQIYNKDFAKGHHGKPNLHTLYWTGLFSPENLAKTSIKLNGQAELFYRPKSRMKRMAHRLGEKMLNKKLKDQKTPIPDTLYQELYDYVNHRLSHDLSDEARALLPNVITKEVSHEIIKDRRFTSDKFFFHVPITLNYQAANSPSKFNQRVNAYLKEHPETPIIGIDRGERNLIYITVIDSTGKILEQRSLNTIQQFDYQKKLDNREKERVAARQAWSVVGTIKDLKQGYLSQVIHEIVDLMIHYQAVVVLENLNFGFKSKRTGIAEKAVYQQFEKMLIDKLNCLVLKDYPAEKVGGVLNPYQLTDQFTSFAKMGTQSGFLFYVPAPYTSKIDPLTGFVDPFVWKTIKNHESRKHFLEGFDFLHYDVKTGDFILHFKMNRNLSFQRGLPGFMPAWDIVFEKNETQFDAKGTPFIAGKRIVPVIENHRFTGRYRDLYPANELIALLEEKGIVFRDGSNILPKLLENDDSHAIDTMVALIRSVLQMRNSNAATGEDYINSPVRDLNGVCFDSRFQNPEWPMDADANGAYHIALKGQLLLNHLKESKDLKLQNGISNQDWLAYIQELRN

SEQ ID NO: 37 - protein, 1300 aa, Francisella tularensis subsp. tularensis
MSIYQEFVNKYSLSKTLRFELIPQGKTLENIKARGLILDDEKRAKDYKKAKQIIDKYHQFFIEEILSSVCISEDLLQNYSDVYFKLKKSDDDNLQKDFKSAKDTIKKQISEYIKDSEKFKNLFNQNLIDAKKGQESDLILWLKQSKDNGIELFKANSDITDIDEALEIIKSFKGWTTYFKGFHENRKNVYSSDDIPTSIIYRIVDDNLPKFLENKAKYESLKDKAPEAINYEQIKKDLAEELTFDIDYKTSEVNQRVFSLDEVFEIANFNNYLNQSGITKFNTIIGGKFVNGENTKRKGINEYINLYSQQINDKTLKKYKMSVLFKQILSDTESKSFVIDKLEDDSDVVTTMQSFYEQIAAFKTVEEKSIKETLSLLFDDLKAQKLDLSKIYFKNDKSLTDLSQQVFDDYSVIGTAVLEYITQQVAPKNLDNPSKKEQDLIAKKTEKAKYLSLETIKLALEEFNKHRDIDKQCRFEEILANFAAIPMIFDEIAQNKDNLAQISLKYQNQGKKDLLQASAEEDVKAIKDLLDQTNNLLHRLKIFHISQSEDKANILDKDEHFYLVFEECYFELANIVPLYNKIRNYITQKPYSDEKFKLNFENSTLANGWDKNKEPDNTAILFIKDDKYYLGVMNKKNNKIFDDKAIKENKGEGYKKIVYKLLPGANKMLPKVFFSAKSIKFYNPSEDILRIRNHSTHTKNGNPQKGYEKFEFNIEDCRKFIDFYKESISKHPEWKDFGFRFSDTQRYNSIDEFYREVENQGYKLTFENISESYIDSVVNQGKLYLFQIYNKDFSAYSKGRPNLHTLYWKALFDERNLQDVVYKLNGEAELFYRKQSIPKKITHPAKEAIANKNKDNPKKESVFEYDLIKDKRFTEDKFFFHCPITINFKSSGANKFNDEINLLLKEKANDVHILSIDRGERHLAYYTLVDGKGNIIKQDTFNIIGNDRMKTNYHDKLAAIEKDRDSARKDWKKINNIKEMKEGYLSQVVHEIAKLVIEHNAIVVFEDLNFGFKRGRFKVEKQVYQKLEKMLIEKLNYLVFKDNEFDKTGGVLRAYQLTAPFETFKKMGKQTGIIYYVPAGFTSKICPVTGFVNQLYPKYESVSKSQEFFSKFDKICYNLDKGYFEFSFDYKNFGDKAAKGKWTIASFGSRLINFRNSDKNHNWDTREVYPTKELEKLLKDYSIEYGHGECIKAAICGESDKKFFAKLTSVLNTILQMRNSKTGTELDYLISPVADVNGNFFDSRQAPKNMPQDADANGAYHIGLKGLMLLDRIKNNQEGKKLNLVIKNEEYFEFVQNRNN

SEQ ID NO: 38 - protein, 1388 aa, Streptococcus thermophilus
MTKPYSIGLDIGTNSVGWAVTTDNYKVPSKKMKVLGNTSKKYIKKNLLGVLLFDSGITAEGRRLKRTARRRYTRRRNRILYLQEIFSTEMATLDDAFFQRLDDSFLVPDDKRDSKYPIFGNLVEEKAYHDEFPTIYHLRKYLADSTKKADLRLVYLALAHMIKYRGHFLIEGEFNSKNNDIQKNFQDFLDTYNAIFESDLSLENSKQLEEIVKDKISKLEKKDRILKLFPGEKNSGIFSEFLKLIVGNQADFRKCFNLDEKASLHFSKESYDEDLETLLGYIGDDYSDVFLKAKKLYDAILLSGFLTVTDNETEAPLSSAMIKRYNEHKEDLALLKEYIRNISLKTYNEVFKDDTKNGYAGYIDGKTNQEDFYVYLKKLLAEFEGADYFLEKIDREDFLRKQRTFDNGSIPYQIHLQEMRAILDKQAKFYPFLAKNKERIEKILTFRIPYYVGPLARGNSDFAWSIRKRNEKITPWNFEDVIDKESSAEAFINRMTSFDLYLPEEKVLPKHSLLYETFNVYNELTKVRFIAESMRDYQFLDSKQKKDIVRLYFKDKRKVTDKDIIEYLHAIYGYDGIELKGIEKQFNSSLSTYHDLLNIINDKEFLDDSSNEAIIEEIIHTLTIFEDREMIKQRLSKFENIFDKSVLKKLSRRHYTGWGKLSAKLINGIRDEKSGNTILDYLIDDGISNRNFMQLIHDDALSFKKKIQKAQIIGDEDKGNIKEVVKSLPGSPAIKKGILQSIKIVDELVKVMGGRKPESIVVEMARENQYTNQGKSNSQQRLKRLEKSLKELGSKILKENIPAKLSKIDNNALQNDRLYLYYLQNGKDMYTGDDLDIDRLSNYDIDHIIPQAFLKDNSIDNKVLVSSASNRGKSDDVPSLEVVKKRKTFWYQLLKSKLISQRKFDNLTKAERGGLSPEDKAGFIQRQLVETRQITKHVARLLDEKFNNKKDENNRAVRTVKIITLKSTLVSQFRKDFELYKVREINDFHHAHDAYLNAVVASALLKKYPKLEPEFVYGDYPKYNSFRERKSATEKVYFYSNIMNIFKKSISLADGRVIERPLIEVNEETGESVWNKESDLATVRRVLSYPQVNVVKKVEEQNHGLDRGKPKGLFNANLSSKPKPNSNENLVGAKEYLDPKKYGGYAGISNSFTVLVKGTIEKGAKKKITNVLEFQGISILDRINYRKDKLNFLLEKGYKDIELIIELPKYSLFELSDGSRRMLASILSTNNKRGEIHKGNQIFLSQKFVKLLYHAKRISNTINENHRKYVENHKKEFEELFYYILEFNENYVGAKKNGKLLNSAFQSWQNHSIDELCSSFIGPTGSERKGLFELTSRGSAADFEFLGVKIPRYRDYTPSSLLKDATLIHQSVTGLYETRIDLAKLGEG

SEQ ID NO: 39 - protein, 1400 aa, Artificial sequence
  GenBank: AKE81023.1 Cas9 [Plant multiplex genome editing vector pYLCRISPR/Cas9P35s-B]
MAPKKKRKVGIHGVPAADKKYSIGLDIGTNSVGWAVITDEYKVPSKKFKVLGNTDRHSIKKNLIGALLFDSGETAEATRLKRTARRRYTRRKNRICYLQEIFSNEMAKVDDSFFHRLEESFLVEEDKKHERHPIFGNIVDEVAYHEKYPTIYHLRKKLVDSTDKADLRLIYLALAHMIKFRGHFLIEGDLNPDNSDVDKLFIQLVQTYNQLFEENPINASGVDAKAILSARLSKSRRLENLIAQLPGEKKNGLFGNLIALSLGLTPNFKSNFDLAEDAKLQLSKDTYDDDLDNLLAQIGDQYADLFLAAKNLSDAILLSDILRVNTEITKAPLSASMIKRYDEHHQDLTLLKALVRQQLPEKYKEIFFDQSKNGYAGYIDGGASQEEFYKFIKPILEKMDGTEELLVKLNREDLLRKQRTFDNGSIPHQIHLGELHAILRRQEDFYPFLKDNREKIEKILTFRIPYYVGPLARGNSRFAWMTRKSEETITPWNFEEVVDKGASAQSFIERMTNFDKNLPNEKVLPKHSLLYEYFTVYNELTKVKYVTEGMRKPAFLSGEQKKAIVDLLFKTNRKVTVKQLKEDYFKKIECFDSVEISGVEDRFNASLGTYHDLLKIIKDKDFLDNEENEDILEDIVLTLTLFEDREMIEERLKTYAHLFDDKVMKQLKRRRYTGWGRLSRKLINGIRDKQSGKTILDFLKSDGFANRNFMQLIHDDSLTFKEDIQKAQVSGQGDSLHEHIANLAGSPAIKKGILQTVKVVDELVKVMGRHKPENIVIEMARENQTTQKGQKNSRERMKRIEEGIKELGSQILKEHPVENTQLQNEKLYLYYLQNGRDMYVDQELDINRLSDYDVDHIVPQSFLKDDSIDNKVLTRSDKNRGKSDNVPSEEVVKKMKNYWRQLLNAKLITQRKFDNLTKAERGGLSELDKAGFIKRQLVETRQITKHVAQILDSRMNTKYDENDKLIREVKVITLKSKLVSDFRKDFQFYKVREINNYHHAHDAYLNAVVGTALIKKYPKLESEFVYGDYKVYDVRKMIAKSEQEIGKATAKYFFYSNIMNFFKTEITLANGEIRKRPLIETNGETGEIVWDKGRDFATVRKVLSMPQVNIVKKTEVQTGGFSKESILPKRNSDKLIARKKDWDPKKYGGFDSPTVAYSVLVVAKVEKGKSKKLKSVKELLGITIMERSSFEKNPIDFLEAKGYKEVKKDLIIKLPKYSLFELENGRKRMLASAGELQKGNELALPSKYVNFLYLASHYEKLKGSPEDNEQKQLFVEQHKHYLDEIIEQISEFSKRVILADANLDKVLSAYNKHRDKPIREQAENIIHLFTLTNLGAPAAFKYFDTTIDRKRYTSTKEVLDATLIHQSITGLYETRIDLSQLGGDKRPAATKKAGQAKKKK

SEQ ID NO: 40 - protein, 1053 aa, Staphylococcus aureus
MKRNYILGLDIGITSVGYGIIDYETRDVIDAGVRLFKEANVENNEGRRSKRGARRLKRRRRHRIQRVKKLLFDYNLLTDHSELSGINPYEARVKGLSQKLSEEEFSAALLHLAKRRGVHNVNEVEEDTGNELSTKEQISRNSKALEEKYVAELQLERLKKDGEVRGSINRFKTSDYVKEAKQLLKVQKAYHQLDQSFIDTYIDLLETRRTYYEGPGEGSPFGWKDIKEWYEMLMGHCTYFPEELRSVKYAYNADLYNALNDLNNLVITRDENEKLEYYEKFQIIENVFKQKKKPTLKQIAKEILVNEEDIKGYRVTSTGKPEFTNLKVYHDIKDITARKEIIENAELLDQIAKILTIYQSSEDIQEELTNLNSELTQEEIEQISNLKGYTGTHNLSLKAINLILDELWHTNDNQIAIFNRLKLVPKKVDLSQQKEIPTTLVDDFILSPVVKRSFIQSIKVINAIIKKYGLPNDIIIELAREKNSKDAQKMINEMQKRNRQTNERIEEIIRTTGKENAKYLIEKIKLHDMQEGKCLYSLEAIPLEDLLNNPFNYEVDHIIPRSVSFDNSFNNKVLVKQEENSKKGNRTPFQYLSSSDSKISYETFKKHILNLAKGKGRISKTKKEYLLEERDINRFSVQKDFINRNLVDTRYATRGLMNLLRSYFRVNNLDVKVKSINGGFTSFLRRKWKFKKERNKGYKHHAEDALIIANADFIFKEWKKLDKAKKVMENQMFEEKQAESMPEIETEQEYKEIFITPHQIKHIKDFKDYKYSHRVDKKPNRELINDTLYSTRKDDKGNTLIVNNLNGLYDKDNDKLKKLINKSPEKLLMYHHDPQTYQKLKLIMEQYGDEKNPLYKYYEETGNYLTKYSKKDNGPVIKKIKYYGNKLNAHLDITDDYPNSRNKVVKLSLKPYRFDVYLDNGVYKFVTVKNLDVIKKENYYEVNSKCYEEAKKLKKISNQAEFIASFYNNDLIKINGELYRVIGVNNDLLNRIEVNMIDITYREYLENMNDKRPPRIIKTIASKTQSIKKYSTDILGNLYEVKSKKHPQIIKKG

SEQ ID NO: 41 - protein, 1368 aa, Artificial sequence
  Nuclease deficient Cas9 GenBank: AKA60242.1
MDKKYSIGLAIGTNSVGWAVITDEYKVPSKKFKVLGNTDRHSIKKNLIGALLFDSGETAEATRLKRTARRRYTRRKNRICYLQEIFSNEMAKVDDSFFHRLEESFLVEEDKKHERHPIFGNIVDEVAYHEKYPTIYHLRKKLVDSTDKADLRLIYLALAHMIKFRGHFLIEGDLNPDNSDVDKLFIQLVQTYNQLFEENPINASGVDAKAILSARLSKSRRLENLIAQLPGEKKNGLFGNLIALSLGLTPNFKSNFDLAEDAKLQLSKDTYDDDLDNLLAQIGDQYADLFLAAKNLSDAILLSDILRVNTEITKAPLSASMIKRYDEHHQDLTLLKALVRQQLPEKYKEIFFDQSKNGYAGYIDGGASQEEFYKFIKPILEKMDGTEELLVKLNREDLLRKQRTFDNGSIPHQIHLGELHAILRRQEDFYPFLKDNREKIEKILTFRIPYYVGPLARGNSRFAWMTRKSEETITPWNFEEVVDKGASAQSFIERMTNFDKNLPNEKVLPKHSLLYEYFTVYNELTKVKYVTEGMRKPAFLSGEQKKAIVDLLFKTNRKVTVKQLKEDYFKKIECFDSVEISGVEDRFNASLGTYHDLLKIIKDKDFLDNEENEDILEDIVLTLTLFEDREMIEERLKTYAHLFDDKVMKQLKRRRYTGWGRLSRKLINGIRDKQSGKTILDFLKSDGFANRNFMQLIHDDSLTFKEDIQKAQVSGQGDSLHEHIANLAGSPAIKKGILQTVKVVDELVKVMGRHKPENIVIEMARENQTTQKGQKNSRERMKRIEEGIKELGSQILKEHPVENTQLQNEKLYLYYLQNGRDMYVDQELDINRLSDYDVDAIVPQSFLKDDSIDNKVLTRSDKNRGKSDNVPSEEVVKKMKNYWRQLLNAKLITQRKFDNLTKAERGGLSELDKAGFIKRQLVETRQITKHVAQILDSRMNTKYDENDKLIREVKVITLKSKLVSDFRKDFQFYKVREINNYHHAHDAYLNAVVGTALIKKYPKLESEFVYGDYKVYDVRKMIAKSEQEIGKATAKYFFYSNIMNFFKTEITLANGEIRKRPLIETNGETGEIVWDKGRDFATVRKVLSMPQVNIVKKTEVQTGGFSKESILPKRNSDKLIARKKDWDPKKYGGFDSPTVAYSVLVVAKVEKGKSKKLKSVKELLGITIMERSSFEKNPIDFLEAKGYKEVKKDLIIKLPKYSLFELENGRKRMLASAGELQKGNELALPSKYVNFLYLASHYEKLKGSPEDNEQKQLFVEQHKHYLDEIIEQISEFSKRVILADANLDKVLSAYNKHRDKPIREQAENIIHLFTLTNLGAPAAFKYFDTTIDRKRYTSTKEVLDATLIHQSITGLYETRIDLSQLGGD

SEQ ID NO: 42 - DNA, 363 bp, Artificial sequence
  mSA variant
gcggaagcgggtatcaccggcacgtggtacaaccagcatggttctaccttcaccgttaccgcgggtgcggacggtaacctgaccggtcagtacgaaaaccgtgcgcagggcactggttgccagaactctccgtacaccctgaccggtcgttacaacggtaccaaactggaatggcgtgttgaatggaacaactctaccgaaaactgccactctcgtaccgaatggcgtggtcagtaccagggtggtgcggaagcgcgtatcaacacccagtggaacctgacctacgaaggtggttctggtccggcgaccgaacagggtcaggacaccttcaccaaagttaaaccgtctgcggcgtctggatcc

SEQ ID NO: 43 - DNA, 714 bp, Artificial sequence
  scFv fluorescein variant
caggtccagctccaagagtctggtggggatctggttaaaccgggcggaagcttgaagctttcatgtgccgcgtcaggatttactttctctggttatggtatgtcttgggtgagacaaacgcctgataaaagactggagcaagtggcgtctatatcacgggatgggtacacgacctattatactgattcagttaaagggcgcttcactatatcacgcgataatgctaggaacacgctgtacctccagatgtcttcactgcagtccgctgacaccgccatctattattgcgcaaggttgggaacctattggggacaagggactactgttaccgtgtcctccggcggtggggggtccggaggaagggcctctggcggtggtggctcccagattgtgttgactcagagccctgctattatgtctgcgtctccgggggagaaagttacaatgacgtgtagagcgtcgtcgtcggtgtcttacatgcactggtatcagctgaagtctggcacatcgcccaaacgctggatttatgatacctcgaaacttagctcaggagttccgactcggttctctggttccgggtctgggacatcgtattccttgactatatcctctatggaagctcatgacgccgcaacatattactgtcaacaatggaactcgaaacctcctttcacctttggttcgggcactaaattggaaataaagcgggccgcc

SEQ ID NO: 44 - DNA, 4587 bp, Artificial sequence
  Cas variant - mSA variant fusion construct
atggataagaagtactctatcggactcgatatcggaactaactctgtgggatgggctgtgatcaccgatgagtacaaggtgccatctaagaagttcaaggttctcggaaacaccgataggcactctatcaagaaaaaccttatcggtgctctcctcttcgattctggtgaaactgctgaggctaccagactcaagagaaccgctagaagaaggtacaccagaagaaagaacaggatctgctacctccaagagatcttctctaacgagatggctaaagtggatgattcattcttccacaggctcgaagagtcattcctcgtggaagaagataagaagcacgagaggcaccctatcttcggaaacatcgttgatgaggtggcataccacgagaagtaccctactatctaccacctcagaaagaagctcgttgattctactgataaggctgatctcaggctcatctacctcgctctcgctcacatgatcaagttcagaggacacttcctcatcgagggtgatctcaaccctgataactctgatgtggataagttgttcatccagctcgtgcagacctacaaccagcttttcgaagagaaccctatcaacgcttcaggtgtggatgctaaggctatcctctctgctaggctctctaagtcaagaaggcttgagaacctcattgctcagctccctggtgagaagaagaacggacttttcggaaacttgatcgctctctctctcggactcacccctaacttcaagtctaacttcgatctcgctgaggatgcaaagctccagctctcaaaggatacctacgatgatgatctcgataacctcctcgctcagatcggagatcagtacgctgatttgttcctcgctgctaagaacctctctgatgctatcctcctcagtgatatcctcagagtgaacaccgagatcaccaaggctccactctcagcttctatgatcaagagatacgatgagcaccaccaggatctcacacttctcaaggctcttgttagacagcagctcccagagaagtacaaagagattttcttcgatcagtctaagaacggatacgctggttacatcgatggtggtgcatctcaagaagagttctacaagttcatcaagcctatcctcgagaagatggatggaaccgaggaactcctcgtgaagctcaatagagaggatcttctcagaaagcagaggaccttcgataacggatctatccctcatcagatccacctcggagagttgcacgctatccttagaaggcaagaggatttctacccattcctcaaggataacagggaaaagattgagaagattctcaccttcagaatcccttactacgtgggacctctcgctagaggaaactcaagattcgcttggatgaccagaaagtctgaggaaaccatcaccccttggaacttcgaagaggtggtggataagggtgctagtgctcagtctttcatcgagaggatgaccaacttcgataagaaccttccaaacgagaaggtgctccctaagcactctttgctctacgagtacttcaccgtgtacaacgagttgaccaaggttaagtacgtgaccgagggaatgaggaagcctgcttttttgtcaggtgagcaaaagaaggctatcgttgatctcttgttcaagaccaacagaaaggtgaccgtgaagcagctcaaagaggattacttcaagaaaatcgagtgcttcgattcagttgagatttctggtgttgaggataggttcaacgcatctctcggaacctaccacgatctcctcaagatcattaaggataaggatttcttggataacgaggaaaacgaggatatcttggaggatatcgttcttaccctcaccctctttgaagatagagagatgattgaagaaaggctcaagacctacgctcatctcttcgatgataaggtgatgaagcagttgaagagaagaagatacactggttggggaaggctctcaagaaagctcattaacggaatcagggataagcagtctggaaagacaatccttgatttcctcaagtctgatggattcgctaacagaaacttcatgcagctcatccacgatgattctctcacctttaaagaggatatccagaaggctcaggtttcaggacagggtgatagtctccatgagcatatcgctaacctcgctggatctcctgcaatcaagaagggaatcctccagactgtgaaggttgtggatgagttggtgaaggtgatgggaaggcataagcctgagaacatcgtgatcgaaatggctagagagaaccagaccactcagaagggacagaagaactctagggaaaggatgaagaggatcgaggaaggtatcaaagagcttggatctcagatcctcaaagagcaccctgttgagaacactcagctccagaatgagaagctctacctctactacctccagaacggaagggatatgtatgtggatcaagagttggatatcaacaggctctctgattacgatgttgatcatatcgtgccacagtcattcttgaaggatgattctatcgataacaaggtgctcaccaggtctgataagaacaggggtaagagtgataacgtgccaagtgaagaggttgtgaagaaaatgaagaactattggaggcagctcctcaacgctaagctcatcactcagagaaagttcgataacttgactaaggctgagaggggaggactctctgaattggataaggcaggattcatcaagaggcagcttgtggaaaccaggcagatcactaagcacgttgcacagatcctcgattctaggatgaacaccaagtacgatgagaacgataagttgatcagggaagtgaaggttatcaccctcaagtcaaagctcgtgtctgatttcagaaaggatttccaattctacaaggtgagggaaatcaacaactaccaccacgctcacgatgcttaccttaacgctgttgttggaaccgctctcatcaagaagtatcctaagctcgagtcagagttcgtgtacggtgattacaaggtgtacgatgtgaggaagatgatcgctaagtctgagcaagagatcggaaaggctaccgctaagtatttcttctactctaacatcatgaatttcttcaagaccgagattaccctcgctaacggtgagatcagaaagaggccactcatcgagacaaacggtgaaacaggtgagatcgtgtgggataagggacgcgacttcgcaaccgtgaggaaggtgctgtccatgccccaggtcaatatagtgaagaaaacggaagttcaaactggtggattttccaaggagtctattctgccgaaacggaattctgataagctgatagcaagaaaaaaagactgggatcctaagaagtatggcggtttcgatagcccaacggtcgcgtactcggtcctcgtcgttgcaaaggttgaaaagggtaagtccaaaaaactgaagtcggtgaaggagttgctcggtatcactatcatggaaaggtcttcttttgaaaagaacccgatcgacttcctcgaagctaaaggctataaagaggttaagaaggacctcataattaaactgcccaagtactcacttttcgaattggagaacgggagaaagagaatgctcgcttctgctggtgagcttcaaaagggaaacgagcttgctctcccatctaagtacgttaactttctttacctcgcttctcactacgagaagttgaagggatctccagaagataacgagcagaagcaacttttcgttgagcagcacaagcactacttggatgagatcatcgagcagatctctgagttctctaaaagggtgatcctcgctgatgcaaacctcgataaggtgttgtctgcttacaacaagcacagagataagcctatcagggaacaggcagagaacatcatccatctcttcacccttaccaacctcggtgctcctgctgctttcaagtacttcgatacaaccatcgataggaagagatacacctctaccaaagaagtgctcgatgctaccctcatccatcagtctatcactggactctacgagactaggatcgatctctcacagctcggtggtgattcaagggctgatcctaagaagaagaggaaggttcatcaccatcaccatcaccatcaccatcacaaagaatccggtagcgtttcttcggaacagctggcccagttccgcagcctggatgcggaagcgggtatcaccggcacgtggtacaaccagcatggttctaccttcaccgttaccgcgggtgcggacggtaacctgaccggtcagtacgaaaaccgtgcgcagggcactggttgccagaactctccgtacaccctgaccggtcgttacaacggtaccaaactggaatggcgtgttgaatggaacaactctaccgaaaactgccactctcgtaccgaatggcgtggtcagtaccagggtggtgcggaagcgcgtatcaacacccagtggaacctgacctacgaaggtggttctggtccggcgaccgaacagggtcaggacaccttcaccaaagttaaaccgtctgcggcgtctggatcctaa

SEQ ID NO: 45 - DNA, 4938 bp, Artificial sequence
  Cas variant - scFv (fluorescein) fusion construct
atggataagaagtactctatcggactcgatatcggaactaactctgtgggatgggctgtgatcaccgatgagtacaaggtgccatctaagaagttcaaggttctcggaaacaccgataggcactctatcaagaaaaaccttatcggtgctctcctcttcgattctggtgaaactgctgaggctaccagactcaagagaaccgctagaagaaggtacaccagaagaaagaacaggatctgctacctccaagagatcttctctaacgagatggctaaagtggatgattcattcttccacaggctcgaagagtcattcctcgtggaagaagataagaagcacgagaggcaccctatcttcggaaacatcgttgatgaggtggcataccacgagaagtaccctactatctaccacctcagaaagaagctcgttgattctactgataaggctgatctcaggctcatctacctcgctctcgctcacatgatcaagttcagaggacacttcctcatcgagggtgatctcaaccctgataactctgatgtggataagttgttcatccagctcgtgcagacctacaaccagcttttcgaagagaaccctatcaacgcttcaggtgtggatgctaaggctatcctctctgctaggctctctaagtcaagaaggcttgagaacctcattgctcagctccctggtgagaagaagaacggacttttcggaaacttgatcgctctctctctcggactcacccctaacttcaagtctaacttcgatctcgctgaggatgcaaagctccagctctcaaaggatacctacgatgatgatctcgataacctcctcgctcagatcggagatcagtacgctgatttgttcctcgctgctaagaacctctctgatgctatcctcctcagtgatatcctcagagtgaacaccgagatcaccaaggctccactctcagcttctatgatcaagagatacgatgagcaccaccaggatctcacacttctcaaggctcttgttagacagcagctcccagagaagtacaaagagattttcttcgatcagtctaagaacggatacgctggttacatcgatggtggtgcatctcaagaagagttctacaagttcatcaagcctatcctcgagaagatggatggaaccgaggaactcctcgtgaagctcaatagagaggatcttctcagaaagcagaggaccttcgataacggatctatccctcatcagatccacctcggagagttgcacgctatccttagaaggcaagaggatttctacccattcctcaaggataacagggaaaagattgagaagattctcaccttcagaatcccttactacgtgggacctctcgctagaggaaactcaagattcgcttggatgaccagaaagtctgaggaaaccatcaccccttggaacttcgaagaggtggtggataagggtgctagtgctcagtctttcatcgagaggatgaccaacttcgataagaaccttccaaacgagaaggtgctccctaagcactctttgctctacgagtacttcaccgtgtacaacgagttgaccaaggttaagtacgtgaccgagggaatgaggaagcctgcttttttgtcaggtgagcaaaagaaggctatcgttgatctcttgttcaagaccaacagaaaggtgaccgtgaagcagctcaaagaggattacttcaagaaaatcgagtgcttcgattcagttgagatttctggtgttgaggataggttcaacgcatctctcggaacctaccacgatctcctcaagatcattaaggataaggatttcttggataacgaggaaaacgaggatatcttggaggatatcgttcttaccctcaccctctttgaagatagagagatgattgaagaaaggctcaagacctacgctcatctcttcgatgataaggtgatgaagcagttgaagagaagaagatacactggttggggaaggctctcaagaaagctcattaacggaatcagggataagcagtctggaaagacaatccttgatttcctcaagtctgatggattcgctaacagaaacttcatgcagctcatccacgatgattctctcacctttaaagaggatatccagaaggctcaggtttcaggacagggtgatagtctccatgagcatatcgctaacctcgctggatctcctgcaatcaagaagggaatcctccagactgtgaaggttgtggatgagttggtgaaggtgatgggaaggcataagcctgagaacatcgtgatcgaaatggctagagagaaccagaccactcagaagggacagaagaactctagggaaaggatgaagaggatcgaggaaggtatcaaagagcttggatctcagatcctcaaagagcaccctgttgagaacactcagctccagaatgagaagctctacctctactacctccagaacggaagggatatgtatgtggatcaagagttggatatcaacaggctctctgattacgatgttgatcatatcgtgccacagtcattcttgaaggatgattctatcgataacaaggtgctcaccaggtctgataagaacaggggtaagagtgataacgtgccaagtgaagaggttgtgaagaaaatgaagaactattggaggcagctcctcaacgctaagctcatcactcagagaaagttcgataacttgactaaggctgagaggggaggactctctgaattggataaggcaggattcatcaagaggcagcttgtggaaaccaggcagatcactaagcacgttgcacagatcctcgattctaggatgaacaccaagtacgatgagaacgataagttgatcagggaagtgaaggttatcaccctcaagtcaaagctcgtgtctgatttcagaaaggatttccaattctacaaggtgagggaaatcaacaactaccaccacgctcacgatgcttaccttaacgctgttgttggaaccgctctcatcaagaagtatcctaagctcgagtcagagttcgtgtacggtgattacaaggtgtacgatgtgaggaagatgatcgctaagtctgagcaagagatcggaaaggctaccgctaagtatttcttctactctaacatcatgaatttcttcaagaccgagattaccctcgctaacggtgagatcagaaagaggccactcatcgagacaaacggtgaaacaggtgagatcgtgtgggataagggacgcgacttcgcaaccgtgaggaaggtgctgtccatgccccaggtcaatatagtgaagaaaacggaagttcaaactggtggattttccaaggagtctattctgccgaaacggaattctgataagctgatagcaagaaaaaaagactgggatcctaagaagtatggcggtttcgatagcccaacggtcgcgtactcggtcctcgtcgttgcaaaggttgaaaagggtaagtccaaaaaactgaagtcggtgaaggagttgctcggtatcactatcatggaaaggtcttcttttgaaaagaacccgatcgacttcctcgaagctaaaggctataaagaggttaagaaggacctcataattaaactgcccaagtactcacttttcgaattggagaacgggagaaagagaatgctcgcttctgctggtgagcttcaaaagggaaacgagcttgctctcccatctaagtacgttaactttctttacctcgcttctcactacgagaagttgaagggatctccagaagataacgagcagaagcaacttttcgttgagcagcacaagcactacttggatgagatcatcgagcagatctctgagttctctaaaagggtgatcctcgctgatgcaaacctcgataaggtgttgtctgcttacaacaagcacagagataagcctatcagggaacaggcagagaacatcatccatctcttcacccttaccaacctcggtgctcctgctgctttcaagtacttcgatacaaccatcgataggaagagatacacctctaccaaagaagtgctcgatgctaccctcatccatcagtctatcactggactctacgagactaggatcgatctctcacagctcggtggtgattcaagggctgatcctaagaagaagaggaaggttcatcaccatcaccatcaccatcaccatcacaaagaatccggtagcgtttcttcggaacagctggcccagttccgcagcctggatcaggtccagctccaagagtctggtggggatctggttaaaccgggcggaagcttgaagctttcatgtgccgcgtcaggatttactttctctggttatggtatgtcttgggtgagacaaacgcctgataaaagactggagcaagtggcgtctatatcacgggatgggtacacgacctattatactgattcagttaaagggcgcttcactatatcacgcgataatgctaggaacacgctgtacctccagatgtcttcactgcagtccgctgacaccgccatctattattgcgcaaggttgggaacctattggggacaagggactactgttaccgtgtcctccggcggtggggggtccggaggaagggcctctggcggtggtggctcccagattgtgttgactcagagccctgctattatgtctgcgtctccgggggagaaagttacaatgacgtgtagagcgtcgtcgtcggtgtcttacatgcactggtatcagctgaagtctggcacatcgcccaaacgctggatttatgatacctcgaaacttagctcaggagttccgactcggttctctggttccgggtctgggacatcgtattccttgactatatcctctatggaagctcatgacgccgcaacatattactgtcaacaatggaactcgaaacctcctttcacctttggttcgggcactaaattggaaataaagcgggccgcctaa

SEQ ID NO: 46 - DNA, 2769 bp, Artificial sequence
  NgAgo construct
atggcgtcctccccaaagaagaagcgtaaggtcatgactgttatcgaccttgattctactacaaccgctgacgaacttacttccggacacacctacgacatttcggttactcttaccggcgtttacgacaatactgatgagcaacaccccaggatgtcccttgcattcgaacaagacaacggcgagagaaggtacatcactctgtggaaaaacactacacctaaggacgtgttcacctacgattacgcaaccgggagtacatacatctttacaaacatcgactacgaggtaaaggacgggtacgaaaacctaacagctacttaccagaccactgtcgagaatgctacagcccaagaggtgggcaccaccgacgaggatgaaacattcgccggaggtgaacctctggaccatcaccttgatgatgctttaaacgaaacccctgacgatgcagagactgagtccgactccggacacgtgatgacttcctttgcatctagggatcagctacctgagtggactcttcacacctacaccctgacagctactgacggagccaaaaccgatactgagtacgccaggcgtacccttgcttacacagtcagacaagaactatacactgaccatgatgccgctccagtcgctaccgatggactgatgcttcttacacctgaaccactgggcgaaacaccacttgaccttgattgcggcgtgagggtggaagccgacgaaactcgcacactggactacaccaccgctaaagatcggttactcgccagagagcttgtagaagagggacttaaacgtagtttatgggacgattaccttgttagaggtatcgacgaggtcctcagtaaggaacctgtccttacctgcgacgagtttgatcttcatgagaggtacgacctttctgtggaagtcggacattcggggagggcataccttcatattaacttccgtcatcgttttgtacctaaactaacactggctgacatcgacgatgacaacatttacccaggacttcgtgtcaaaacaacctaccggccccgtcgtggtcacattgtctggggacttcgggacgagtgcgcaacagactctcttaataccctcggaaaccaaagtgttgtggcttaccataggaacaaccaaacaccaattaacactgaccttctcgacgctatcgaagccgctgatcgccgggttgtggagacacgtagacaaggtcatggggacgacgctgtgtccttcccacaagagcttctggctgttgaacccaacacccatcagatcaagcaattcgcttccgatggcttccatcaacaagccaggtctaagacacgtctttcggcttctcggtgctccgagaaagcccaagcatttgctgaacgtcttgaccctgtccgtcttaacggctctactgtcgagtttagttccgagttcttcaccggaaacaatgaacagcaactgagacttctctacgaaaatggggaatcggtccttacatttcgtgatggagccaggggagcccatccagatgagacattctcgaaaggcattgtaaatccacccgaatcctttgaagtcgctgtcgtccttcctgaacaacaggctgatacctgcaaggctcagtgggacaccatggctgatctactcaaccaagcaggcgctcctcctacaaggagtgaaacagtccagtacgatgccttctccagtcccgagagtattagtcttaacgttgctggagccattgacccatccgaggtggatgccgctttcgtggtacttccaccagaccaagaaggattcgctgacctggcttccccaacagagacatacgacgaactgaaaaaggctcttgctaacatgggaatctacagtcaaatggcttacttcgaccgttttcgcgacgctaaaatcttctacacccgtaatgtcgcccttggcctgcttgcagccgctggaggtgtcgcatttacaacagaacatgctatgcctggagatgctgacatgtttatcgggatcgacgtttccaggtcttaccctgaagatggagccagcggacaaatcaacatcgcagctactgcaaccgctgtctacaaggacggaaccatccttggacacagttccactcgtccacaattaggagaaaaacttcaatccaccgatgtcagggatattatgaagaacgccatcctcggataccaacaagtgaccggagaatctcctacccacattgtgattcatcgtgacggcttcatgaacgaggacttagatcctgccacagagtttctaaacgaacaaggcgtcgagtacgatatcgttgaaattcgcaagcaacctcaaaccaggctattagccgtaagtgatgttcaatacgacacacctgtcaagtccattgctgctatcaaccaaaacgaaccacgcgctaccgtggccacctttggcgcccctgagtaccttgctacacgcgatggtggcggcttacctagacctattcaaatcgagcgcgtcgctggagaaacagatatcgaaactcttacaaggcaagtgtaccttctttctcagagtcacatccaggtccataactccaccgctcggctccctatcacaactgcctacgctgaccaggcttcgacccatgctacaaaaggatacttagtccaaaccggagcctttgaatccaacgtggggttcctgaagcgccctgctgccaccaaaaaggctggacaagccaaaaaaaagaagtacccatacgatgtaccagattacgct

SEQ ID NO: 47 - DNA, 246 bp, Zea mays
tacatcaagtgcaacgactgcggcgtgcgcatcgtggaggccaggtgcgaccgcgacatggccgagtggatccgcgacggcgcgcccggcaggatcaggcagctctgctacgacaaggtgctcggccccgagctcttcttctcgccgctgctctacgtccaggtaaccgtcctccgtacgtcgtcgtagagaggtggagatttttgtggtcggatttctggcatcgctggttgcctgctcccagac

SEQ ID NO: 48 - DNA, 243 bp, Artificial Sequence
  INDEL mutant
tacatcaagtgcaacgactgcggcgtgcgcatcgtggaggccaggtgcgaccgcgacatggccgagtggatccgcgacggcgcgcccggcaggatcaggcagctctgctacgacaaggtgctcggccccgagctcttctcgccgctgctctacgtccaggtaaccgtcctccgtacgtcgtcgtagagaggtggagatttttgtggtcggatttctggcatcgctggttgcctgctcccagac

SEQ ID NO: 49 - DNA, 244 bp, Artificial Sequence
  INDEL mutant
tacatcaagtgcaacgactgcggcgtgcgcatcgtggaggccaggtgcgaccgcgacatggccgagtggatccgcgacggcgcgcccggcaggatcaggcagctctgctacgacaaggtgctcggccccgagcttcttctcgccgctgctctacgtccaggtaaccgtcctccgtacgtcgtcgtagagaggtggagatttttgtggtcggatttctggcatcgctggttgcctgctcccagac

SEQ ID NO: 50 - DNA, 252 bp, Artificial Sequence
  HDR event mutant
tacatcaagtgcaacgactgcggcgtgcgcatcgtggaggccaggtgcgaccgcgacatggccgagtggatccgcgacggcgcgcccggcaggatcaggcagctctgctacgacaagtggtccagcgccgcgacctagctcttcttctcgccgctgctctacgtccaggtaaccgtcctccgtacgtcgtcgtagagaggtggagatttttgtggtcggatttctggcatcgctggttgcctgctcccagac

SEQ ID NO: 51 - DNA, 199 bp, Artificial Sequence
  repair template
cgcatcgtggaggccaggtgcgaccgcgacatggccgagtggatccgcgacggcgcgcccggcaggatcaggcagctctgctacgacaagtggtccagcgccgcgacctagctcttcttctcgccgctgctctacgtccaggtaaccgtcctccgtacgtcgtcgtagagaggtggagatttttgtggtcggatttctg

SEQ ID NO: 52 - DNA, 21 bp, Zea mays
aaggtgctcggccccgagctc

SEQ ID NO: 53 - DNA, 27 bp, Artificial Sequence
  replacing sequence in course of HDR event; sequence encoding KWSSAATL
aagtggtccagcgccgcgacctagctc

SEQ ID NO: 54 - DNA, 717 bp, Artificial Sequence
  scFv fluorescein variant
caggtccagctccaagagtctggtggggatctggttaaaccgggcggaagcttgaagctttcatgtgccgcgtcaggatttactttctctggttatggtatgtcttgggtgagacaaacgcctgataaaagactggagcaagtggcgtctatatcacgggatgggtacacgacctattatactgattcagttaaagggcgcttcactatatcacgcgataatgctaggaacacgctgtacctccagatgtcttcactgcagtccgctgacaccgccatctattattgcgcaaggttgggaacctattggggacaagggactactgttaccgtgtcctccggcggtggggggtccggaggaagggcctctggcggtggtggctcccagattgtgttgactcagagccctgctattatgtctgcgtctccgggggagaaagttacaatgacgtgtagagcgtcgtcgtcggtgtcttacatgcactggtatcagctgaagtctggcacatcgcccaaacgctggatttatgatacctcgaaacttagctcaggagttccgactcggttctctggttccgggtctgggacatcgtattccttgactatatcctctatggaagctcatgacgccgcaacatattactgtcaacaatggaactcgaaacctcctttcacctttggttcgggcactaaattggaaataaagcgggccgcctaa

SEQ ID NO: 55 - DNA, 480 bp, Artificial Sequence
  steptavidin variant
gacccatcgaaagattccaaggcacaggtttcggctgctgaggccggtataaccggaacctggtataaccaactcggatcaacattcatcgtcaccgccggcgcagacggtgctctcaccggtacatacgagtcggcggttgggaacgcagagagccggtacgtcctcacgggccgctacgattctgctcctgcgacagatggtagcggaaccgccttgggttggacggtcgcttggaagaataactaccgcaatgccgactcagctacgacctggagcggccaatatgtgggcggagccgaagccaggattaatacccaatggttgctgacatcaggcaccacggaggccaacgcctggaagtcgaccctggttggtcatgatacctttaccaaggttaaaccatcagccgcatctatagatgcggcaaagaaggcgggggtgaataacggaaatccgcttgatgcagtgcagcaataa

SEQ ID NO: 56 - DNA, 366 bp, Artificial Sequence
  mSA2
gcggaagcgggtatcaccggcacgtggtacaaccagcatggttctaccttcaccgttaccgcgggtgcggacggtaacctgaccggtcagtacgaaaaccgtgcgcagggcactggttgccagaactctccgtacaccctgaccggtcgttacaacggtaccaaactggaatggcgtgttgaatggaacaactctaccgaaaactgccactctcgtaccgaatggcgtggtcagtaccagggtggtgcggaagcgcgtatcaacacccagtggaacctgacctacgaaggtggttctggtccggcgaccgaacagggtcaggacaccttcaccaaagttaaaccgtctgcggcgtctggatcctaa